European Patent Specification EP 3 462 844 B1, published November 27, 2024. Title: PLANT REGULATORY ELEMENTS AND USES THEREOF. Applicant: Monsanto Technology, LLC. The sequence listing filed with the application follows.

SEQUENCE LISTING (10 sequences)

SEQ ID NO: 1 - DNA, 2066 bp, Bouteloua gracilis
  misc_feature (1)..(2066): DNA sequence of a regulatory expression element group comprising a promoter, leader, and intron operably linked and derived from a putative ubiquitin gene from Blue Gama grass.
tacgagcaaacgcacaaccgggatacagatctacggtacagaggttacttccaacgggaaggttcccgtccctctagcgcaagcaagacgacgcagagatggtgaccaaaaacgattctttgctttacctggtcatgacaccaccggatacggataagaaggaaaaccggagcatctctagcaatagagaaatcgacgttgcctcctagaggaagaaagcgacggcctatgcttttttcttttgtcgatgattccactgaattgtttctctatttttttcgttgtgtaatggtcctggtacaaacgttcatccaatcatgcaacttgcaagaataaaaataaaaaatataatctcagacgtccaatcatggcttcctaaaaaaataaaaaggacgagaaactactcagaaaaaataaataaatacacaactgtaggaaccaaagcaaagttgacaaggaaccaaagcaaggcaggtccacatgtgctgcgagcaggtgcgcctcctcctccgtttcttcgccttgctaatcacgtcgctaaatacagaggccgacttaagaatgccgacatggcaattttgctggatatttttgcttccttgtagtatcaaacagaagaatattaacgtgggagtatacagtaattttcttttaccatttttctttaatcgcgtttttgttcaaccaaacacaactttagacgtactagtactccactattttttattttattttctcctacagtacttttgaaaaaaaggaatcttgtcatgcatgattgagatcacggtaacggcgactcacgccgccgcacgggtaacggccaccaaccaaaagtagcaaacggcgtcaacctcctcgacatctccgcgtcgcttttctttttctccgcagagaatgagtggcggggagggaccccacgacgcaaccccacgacgcaaccgcttatcgcagccgggtccacaccgcaccgctgccgtagcgtcatgggactcggcccgcggcccgccctccgacccggacccgctttccttcccctcccgtgtataaataccgccccccctgctcgcctcctccccaatccatccgatccccaatccagtcccgcgagcgaaatcgccgacgaccgatcgaagcgaagcagccttcccccatcctctcaaggtatgcgaattctcgatcctcctctcctatgttcgttgtggatctgctggttaggattgattaggttgtcgtaccatgcctttttcctgttcgtgttcctcagatctatagtcggtttgcacaggtagagggctaatctctagtcgatctgcgggtagagttgttgaatcatgtgctgccttcagttcatgtggtttagatccgtgttgcttgttgcggtcatgtgttcacacaacacgtacggttcctgccgtgcgcggattagccgcgctgaggctctgacgttgtcggtgtgggcgtgatcgcgcgggctgcctaggcttgttattgttgaattaggcttggtcgattgggtctgtttctattcacggatggtcttcgatggttcatgtgcatgctgttggtcgctggttaggtggtgataccgttcgatttttgtttaatctgtctagaattccttagatctgaaattctgtgatgtctacatccagctgcttgttgttgaatattttagctatgttaatctgccatggtcttcgtagtttccatgcataaagccatgcaaatacgttgtatatttactgttgctgcaacccatctcagattctagtttgctgtgtactattaggccttgtaaatgcttgttaaaatggttataaattgtgttcatggttctgtgcctgttaagtcgtcatgtttattttctggctgatgctatctgtgggtagaatttgcataggcttcaatctactgactctatgggtaggatctgtgtagcgttgcatcaaacatggcagtgtcttaatgctttcacataaaatgtggaactgtttatattattattatgtactgcatgttttggtggcctaactttgcctctgctgctaaatttgcaggtgcag

SEQ ID NO: 2 - DNA, 1095 bp, Bouteloua gracilis
  misc_feature (1)..(1095): Promoter sequence derived from a putative ubiquitin gene from Blue Gama grass.
tacgagcaaacgcacaaccgggatacagatctacggtacagaggttacttccaacgggaaggttcccgtccctctagcgcaagcaagacgacgcagagatggtgaccaaaaacgattctttgctttacctggtcatgacaccaccggatacggataagaaggaaaaccggagcatctctagcaatagagaaatcgacgttgcctcctagaggaagaaagcgacggcctatgcttttttcttttgtcgatgattccactgaattgtttctctatttttttcgttgtgtaatggtcctggtacaaacgttcatccaatcatgcaacttgcaagaataaaaataaaaaatataatctcagacgtccaatcatggcttcctaaaaaaataaaaaggacgagaaactactcagaaaaaataaataaatacacaactgtaggaaccaaagcaaagttgacaaggaaccaaagcaaggcaggtccacatgtgctgcgagcaggtgcgcctcctcctccgtttcttcgccttgctaatcacgtcgctaaatacagaggccgacttaagaatgccgacatggcaattttgctggatatttttgcttccttgtagtatcaaacagaagaatattaacgtgggagtatacagtaattttcttttaccatttttctttaatcgcgtttttgttcaaccaaacacaactttagacgtactagtactccactattttttattttattttctcctacagtacttttgaaaaaaaggaatcttgtcatgcatgattgagatcacggtaacggcgactcacgccgccgcacgggtaacggccaccaaccaaaagtagcaaacggcgtcaacctcctcgacatctccgcgtcgcttttctttttctccgcagagaatgagtggcggggagggaccccacgacgcaaccccacgacgcaaccgcttatcgcagccgggtccacaccgcaccgctgccgtagcgtcatgggactcggcccgcggcccgccctccgacccggacccgctttccttcccctcccgtgtataaataccgccccccctgctcgcctcctccccaatccatccgatcccc

SEQ ID NO: 3 - DNA, 69 bp, Bouteloua gracilis
  misc_feature (1)..(69): Leader sequence derived from a putative ubiquitin gene from Blue Gama grass.
aatccagtcccgcgagcgaaatcgccgacgaccgatcgaagcgaagcagccttcccccatcctctcaag

SEQ ID NO: 4 - DNA, 902 bp, Bouteloua gracilis
  misc_feature (1)..(902): Intron sequence derived from a putative ubiquitin gene from Blue Gama grass.
gtatgcgaattctcgatcctcctctcctatgttcgttgtggatctgctggttaggattgattaggttgtcgtaccatgcctttttcctgttcgtgttcctcagatctatagtcggtttgcacaggtagagggctaatctctagtcgatctgcgggtagagttgttgaatcatgtgctgccttcagttcatgtggtttagatccgtgttgcttgttgcggtcatgtgttcacacaacacgtacggttcctgccgtgcgcggattagccgcgctgaggctctgacgttgtcggtgtgggcgtgatcgcgcgggctgcctaggcttgttattgttgaattaggcttggtcgattgggtctgtttctattcacggatggtcttcgatggttcatgtgcatgctgttggtcgctggttaggtggtgataccgttcgatttttgtttaatctgtctagaattccttagatctgaaattctgtgatgtctacatccagctgcttgttgttgaatattttagctatgttaatctgccatggtcttcgtagtttccatgcataaagccatgcaaatacgttgtatatttactgttgctgcaacccatctcagattctagtttgctgtgtactattaggccttgtaaatgcttgttaaaatggttataaattgtgttcatggttctgtgcctgttaagtcgtcatgtttattttctggctgatgctatctgtgggtagaatttgcataggcttcaatctactgactctatgggtaggatctgtgtagcgttgcatcaaacatggcagtgtcttaatgctttcacataaaatgtggaactgtttatattattattatgtactgcatgttttggtggcctaactttgcctctgctgctaaatttgcaggtgcag

SEQ ID NO: 5 - DNA, 498 bp, Bouteloua gracilis
  misc_feature (1)..(498): 3' untranslated region derived from a putative ubiquitin gene from Blue Gama grass.
gtttggtcaggagctgctcttgtctctggtttcacaagtatggtgtctctggtgtatggcgtgtccagtcccgttgtggttcgactgatgtctctgtcgtgttatgagtcctatgtcgtctggttgtccgtgtgaaacattgctgcatgtgcagctaattcgtgtgaaacattgctgcatgtgcagctggttggtttatgaataagtgaaacctgaactttgtgtgaattctgcttcctctatgcgctgaatgttttgattgtgatcttttatctactcacagttgctgagatgataaggctgaatcaatgtagagctaagattctctcgtaaatgtttatattaaataccttgtgtaattgcgagtacaaatcgacagtaattcaagctgcggttctttgttcatccagaaggccaagattgcaaattcaggtttcttggcagtgaaagattgaacgcatgcaaatttcctttgttcttttgatcacaaaattgatc

SEQ ID NO: 6 - DNA, 2001 bp, Artificial
  Synthetic coding sequence encoding Beta-glucuronidase designed for expression in a plant cell.
atggtgaggcccgttgagaccccgactagggagatcaagaagctggacggcctctgggccttctccctcgaccgtgagaactgcggcatcgaccagcgctggtgggagtccgccctccaggagtctagggccatcgccgtgcccggttccttcaacgaccagttcgccgacgccgacatccgcaactacgcgggcaacgtctggtatcagcgcgaggtgttcatcccgaagggctgggcgggccagcgcatcgtgctccgcttcgacgccgtgacccactacggcaaggtctgggtgaacaatcaggaggtaagtttctgcttctacctttgatatatatataataattatcattaattagtagtaatataatatttcaaatatttttttcaaaataaaagaatgtagtatatagcaattgcttttctgtagtttataagtgtgtatattttaatttataacttttctaatatatgaccaaaatttgttgatgtgcaggtgatggagcaccagggcggttacaccccgttcgaggccgacgtgacgccgtacgtgatcgccgggaagtccgtccgcatcaccgtctgcgtgaacaatgagctgaactggcagaccatcccgcctggcatggtcatcaccgacgagaacggcaagaagaagcagtcctacttccacgacttcttcaactacgctggcatccaccgctccgtgatgctctacaccactcccaacacctgggtggacgacatcaccgtggtcacccacgtggcccaggactgcaaccacgcctccgtggactggcaagtcgttgccaacggcgacgtcagcgtcgagctgcgcgacgccgaccagcaagtcgttgccaccggccagggcaccagcggcaccctccaagtcgtcaaccctcacctctggcagcctggcgagggctacctctacgagctgtgcgtcaccgccaagagccagactgagtgcgacatctaccctctccgcgtcggcatcaggagcgtcgctgtcaagggcgagcagttcctcatcaaccacaagcctttctacttcactggtttcggccgccacgaggacgctgacctgaggggcaagggtttcgacaacgtcctgatggtccacgaccacgctctgatggactggatcggtgccaacagctacaggaccagtcactacccgtacgctgaggagatgctggactgggctgacgagcacggtatcgtcgtgatcgacgagactgctgcggtcggtttcaacctgtctctgggcattggtttcgaggctgggaacaagccgaaggagctgtactctgaggaagctgtcaacggcgagactcagcaagctcatctccaggcgattaaggagctgattgccagggacaagaaccatccgtctgtcgtgatgtggtctattgcgaatgagccggacaccagaccgcaaggggcgcgtgaatacttcgcgccgctggcggaggcgactcgcaaactggacccaacccgtccaatcacgtgcgtcaatgtcatgttctgcgacgcccatacggatacgatctcggacctgttcgatgttctttgtctcaatcggtactatgggtggtatgttcagagcggggatcttgagacggcggagaaggttcttgagaaggaactcctggcgtggcaagagaagctccatcagccgatcattatcacggagtacggggttgacacacttgcgggccttcacagtatgtacacagatatgtggtcggaggaataccagtgtgcatggttggatatgtaccatcgtgtcttcgaccgggtttcagcggttgtcggcgaacaagtctggaacttcgcagacttcgccacgagccaagggatactgcgggtaggagggaacaagaagggaatcttcacacgggatcggaagcccaagtcagcagccttcctgttgcagaagcgatggacaggaatgaacttcggagaaaagccacagcaaggcggaaagcagtga

SEQ ID NO: 7 - DNA, 1045 bp, Bouteloua gracilis
  misc_feature (1)..(1045): Enhancer derived from the promoter of a putative ubiquitin gene from Blue Gama grass.
tacgagcaaacgcacaaccgggatacagatctacggtacagaggttacttccaacgggaaggttcccgtccctctagcgcaagcaagacgacgcagagatggtgaccaaaaacgattctttgctttacctggtcatgacaccaccggatacggataagaaggaaaaccggagcatctctagcaatagagaaatcgacgttgcctcctagaggaagaaagcgacggcctatgcttttttcttttgtcgatgattccactgaattgtttctctatttttttcgttgtgtaatggtcctggtacaaacgttcatccaatcatgcaacttgcaagaataaaaataaaaaatataatctcagacgtccaatcatggcttcctaaaaaaataaaaaggacgagaaactactcagaaaaaataaataaatacacaactgtaggaaccaaagcaaagttgacaaggaaccaaagcaaggcaggtccacatgtgctgcgagcaggtgcgcctcctcctccgtttcttcgccttgctaatcacgtcgctaaatacagaggccgacttaagaatgccgacatggcaattttgctggatatttttgcttccttgtagtatcaaacagaagaatattaacgtgggagtatacagtaattttcttttaccatttttctttaatcgcgtttttgttcaaccaaacacaactttagacgtactagtactccactattttttattttattttctcctacagtacttttgaaaaaaaggaatcttgtcatgcatgattgagatcacggtaacggcgactcacgccgccgcacgggtaacggccaccaaccaaaagtagcaaacggcgtcaacctcctcgacatctccgcgtcgcttttctttttctccgcagagaatgagtggcggggagggaccccacgacgcaaccccacgacgcaaccgcttatcgcagccgggtccacaccgcaccgctgccgtagcgtcatgggactcggcccgcggcccgccctccgacccggacccgctttccttcccctcccgtg

SEQ ID NO: 8 - DNA, 300 bp, Oryza sativa
  misc_feature (1)..(300): 3' untranslated region derived from a rice Lipid Transfer Protein-like gene.
attaatcgatcctccgatcccttaattaccataccattacaccatgcatcaatatccatatatatataaaccctttcgcacgtacttatactatgttttgtcatacatatatatgtgtcgaacgatcgatctatcactgatatgatatgattgatccatcagcctgatctctgtatcttgttatttgtataccgtcaaataaaagtttcttccacttgtgttaataattagctactctcatctcatgaaccctatatataactagtttaatttgctgtcaattgaacatgatgatcgatg

SEQ ID NO: 9 - DNA, 631 bp, Artificial
  An enhanced promoter and native leader sequence derived from the Cauliflower mosaic virus.
ggtccgatgtgagacttttcaacaaagggtaatatccggaaacctcctcggattccattgcccagctatctgtcactttattgtgaagatagtggaaaaggaaggtggctcctacaaatgccatcattgcgataaaggaaaggccatcgttgaagatgcctctgccgacagtggtcccaaagatggacccccacccacgaggagcatcgtggaaaaagaagacgttccaaccacgtcttcaaagcaagtggattgatgtgatggtccgatgtgagacttttcaacaaagggtaatatccggaaacctcctcggattccattgcccagctatctgtcactttattgtgaagatagtggaaaaggaaggtggctcctacaaatgccatcattgcgataaaggaaaggccatcgttgaagatgcctctgccgacagtggtcccaaagatggacccccacccacgaggagcatcgtggaaaaagaagacgttccaaccacgtcttcaaagcaagtggattgatgtgatatctccactgacgtaagggatgacgcacaatcccactatccttcgcaagacccttcctctatataaggaagttcatttcatttggagaggacacgctgaacacgctg

SEQ ID NO: 10 - DNA, 253 bp, Agrobacterium tumefaciens
  misc_feature (1)..(253): 3' untranslated region derived from the nopaline synthase gene of Agrobacterium tumefaciens.
gatcgttcaaacatttggcaataaagtttcttaagattgaatcctgttgccggtcttgcgatgattatcatataatttctgttgaattacgttaagcatgtaataattaacatgtaatgcatgacgttatttatgagatgggtttttatgattagagtcccgcaattatacatttaatacgcgatagaaaacaaaatatagcgcgcaaactaggataaattatcgcgcgcggtgtcatctatgttactagatc